European Patent Application EP 4 703 374 A1, published March 4, 2026. Title: Modified Delivery Carrier and Use Thereof. Applicant: 深圳深信生物科技有限公司. The sequence listing filed with the application follows.

SEQUENCE LISTING (12 sequences)

SEQ ID NO: 1 - protein, 5 aa, Synthetic construct
DYGVS

SEQ ID NO: 2 - protein, 16 aa, Synthetic construct
VIWGSETTYYNSALKS

SEQ ID NO: 3 - protein, 13 aa, Synthetic construct
KHYYYGGSYAMDY

SEQ ID NO: 4 - protein, 11 aa, Synthetic construct
RASQDISKYLN

SEQ ID NO: 5 - protein, 7 aa, Synthetic construct
HTSRLHS

SEQ ID NO: 6 - protein, 7 aa, Synthetic construct
GNTLPYT

SEQ ID NO: 7 - protein, 120 aa, Synthetic construct
EVKLQESGPGLVAPSQSLSVTCTVSGVSLPDYGVSWIRQPPRKGLEWLGVIWGSETTYYNSALKSRLTIIKDNSKSQVFLKMNSLQTDDTAIYYCAKHYYYGGSYAMDYWGQGTSVTVSS

SEQ ID NO: 8 - protein, 107 aa, Synthetic construct
DIQMTQTTSSLSASLGDRVTISCRASQDISKYLNWYQQKPDGTVKLLIYHTSRLHSGVPSRFSGSGSGTDYSLTISNLEQEDIATYFCQQGNTLPYTFGGGTKLEIT

SEQ ID NO: 9 - protein, 447 aa, Synthetic construct
EVKLQESGPGLVAPSQSLSVTCTVSGVSLPDYGVSWIRQPPRKGLEWLGVIWGSETTYYNSALKSRLTIIKDNSKSQVFLKMNSLQTDDTAIYYCAKHYYYGGSYAMDYWGQGTSVTVSSASTKGPSVFPLAPCSRSTSESTAALGCLVKDYFPEPVTVSWNSGALTSGVHTFPAVLQSSGLYSLSSVVTVPSSSLGTKTYTCNVDHKPSNTKVDKRVESKYGPPCPPCPAPPVAGGPSVFLFPPKPKDTLMISRTPEVTCVVVAVSQEDPEVQFNWYVDGVEVHNAKTKPREEQFNSTYRVVSVLTVVHQDWLNGKEYKCKVSNKGLPSSIEKTISKAKGQPREPQVYTLPPSQEEMTKNQVSLTCLVKGFYPSDIAVEWESNGQPENNYKTTPPVLDSDGSFFLYSKLTVDKSRWQEGNVFSCSVMHEALHNHYTQKSLSLSLGK

SEQ ID NO: 10 - protein, 214 aa, Synthetic construct
DIQMTQTTSSLSASLGDRVTISCRASQDISKYLNWYQQKPDGTVKLLIYHTSRLHSGVPSRFSGSGSGTDYSLTISNLEQEDIATYFCQQGNTLPYTFGGGTKLEITRTVAAPSVFIFPPSDEQLKSGTASVVCLLNNFYPREAKVQWKVDNALQSGNSQESVTEQDSKDSTYSLSSTLTLSKADYEKHKVYACEVTHQGLSSPVTKSFNRGEC

SEQ ID NO: 11 - DNA, 1341 bp, Synthetic construct
  source 1..1341: mol_type = other DNA
gaagtgaaactgcaggagagcggacctggcctcgtggcccctagccagagcctgagcgtgacctgtaccgtgtccggcgtgtccctgcctgattacggcgtttcttggatccggcagccacccagaaagggcctggaatggctgggcgtcatctggggaagcgagacaacctactacaactctgctctgaaaagcagactgaccatcatcaaggacaatagcaagtcccaggtgttcctgaagatgaacagcctgcaaacagatgacaccgccatctactactgcgccaagcactactactatggcggcagctacgccatggactactggggccagggcaccagcgtgacagtgtctagcgctagcaccaagggccccagcgtgttccccctggccccctgcagccgcagcaccagcgagagcaccgccgccctgggctgcctggtgaaggactacttccccgagcccgtgaccgtgagctggaacagcggcgccctgaccagcggcgtgcacaccttccccgccgtgctgcagagcagcggcctgtacagcctgagcagcgtggtgaccgtgcccagcagcagcctgggcaccaagacctacacctgcaacgtggaccacaagcccagcaacaccaaggtggacaagcgcgtggagagcaagtacggccccccctgccccccctgccccgccccccccgtggccggcggccccagcgtgttcctgttcccccccaagcccaaggacaccctgatgatcagccgcacccccgaggtgacctgcgtggtggtggccgtgagccaggaggaccccgaggtgcagttcaactggtacgtggacggcgtggaggtgcacaacgccaagaccaagccccgcgaggagcagttcaacagcacctaccgcgtggtgagcgtgctgaccgtggtgcaccaggactggctgaacggcaaggagtacaagtgcaaggtgagcaacaagggcctgcccagcagcatcgagaagaccatcagcaaggccaagggccagccccgcgagccccaggtgtacaccctgccccccagccaggaggagatgaccaagaaccaggtgagcctgacctgcctggtgaagggcttctaccccagcgacatcgccgtggagtgggagagcaacggccagcccgagaacaactacaagaccaccccccccgtgctggacagcgacggcagcttcttcctgtacagcaagctgaccgtggacaagagccgctggcaggagggcaacgtgttcagctgcagcgtgatgcacgaggccctgcacaaccactacacccagaagagcctgagcctgagcctgggcaag

SEQ ID NO: 12 - DNA, 642 bp, Synthetic construct
  source 1..642: mol_type = other DNA
gatattcagatgacacagaccacctccagcctctctgctagcctgggcgacagagtgaccatctcttgtagagccagccaggacatcagcaagtacctgaactggtatcagcagaaacctgatggcacagtgaagctgctgatctaccacaccagccggctgcacagcggcgtgcccagcagattcagcggcagcggatctggcaccgactacagcctgacaatctccaacctggagcaggaggacatcgccacctacttctgccagcaaggcaataccctgccttacacctttggcggaggcacaaagctggaaatcacccgtacggtggccgcaccaagcgtcttcatcttcccgccatctgatgagcagttgaaatctggaactgcctctgttgtgtgcctgctgaataacttctatcccagagaggccaaagtacagtggaaggtggataacgccctccaatcgggtaactcccaggagagtgtcacagagcaggacagcaaggacagcacctacagcctcagcagcaccctgacgctgagcaaagcagactacgagaaacacaaagtctacgcctgcgaagtcacccatcagggcctgagctcgcccgtcacaaagagctttaacagaggcgagtgc